European Patent Application EP 4 545 562 A1, published April 30, 2025. Title: FUSION PROTEIN COMPRISING ANTI-CD73 ANTIBODY AND IL-2 AND USE THEREOF. Applicant: GI Innovation, Inc. Application KR. The sequence listing filed with the application follows.

SEQUENCE LISTING (43 sequences)

SEQ ID NO: 1 - protein, 19 aa, synthetic construct
  REGION 1..19: note = mIgG signal
MEWSWVFLFFLSVTTGVHS

SEQ ID NO: 2 - protein, 126 aa, synthetic construct
  REGION 1..126: note = anti-hCD73 sdAb(AHF10235)
QVQVQESGGGLVQAGDSLRLSCAASGRSISRYNMGWFRQAPGKEREFVAAISRSGGVTYYADSVKGRLTISRDNAKSAVYLQMNSLKPEDTAVYYCAADWRNSDSPSPLIIVYDYWGQGTQVTVSS

SEQ ID NO: 3 - protein, 126 aa, synthetic construct
  REGION 1..126: note = anti-hCD73 sdAb(AHF10240)
EVQLVESGGGVVQTGGSLRLSCAASGRTFTHLAMGWFRQAPGKEREFVAAISNSGAGTQFADSVKGRFTISRDNAKNTVYLQMNSLKPEDTAVYYCAADWGTRDSPSKLNAVYDYWGRGTQVTVSS

SEQ ID NO: 4 - protein, 126 aa, synthetic construct
  REGION 1..126: note = anti-hCD73 sdAb(AHP04167)
EVQLVESGGGLVQAGGSLRLSCVVSGRTFSNYHMGWFRQAPGKEREFVAVIGRSGGPTYYADSVKGRFTISRDNAKNTVYLQMNSLKPEDTAVYYCAGDWRNSDSPSKLKPVYDYWGQGTQVTVSS

SEQ ID NO: 5 - protein, 18 aa, synthetic construct
  REGION 1..18: note = Linker 1
GGGGSAESKYGPPCPPCP

SEQ ID NO: 6 - protein, 216 aa, synthetic construct
  REGION 1..216: note = hIgG4 Fc (F01)
APEAAGGPSVFLFPPKPKDQLMISRTPEVTCVVVDVSQEDPEVQFNWYVDGVEVHNAKTKPREEQFNSTYRVVSVLTVLHQDWLNGKEYKCKVSNKGLPSSIEKTISKAKGQPREPQVYTLPPSQEEMTKNQVSLTCLVKGFYPSDIAVEWESNGQPENNYKTTPPVLDSDGSFFLYSRLTVDKSRWQEGNVFSCSVLHEALHNHYTQKSLSLSLG

SEQ ID NO: 7 - protein, 15 aa, synthetic construct
  REGION 1..15: note = Linker 2
GGGGSGGGGSGGGGS

SEQ ID NO: 8 - protein, 133 aa, synthetic construct
  REGION 1..133: note = hIL2v3
APTSSSTKKTQLQLEHLLLDLQMILNGINNYKNPKLTAMLTAKFYMPKKATELKHLQCLERELKPLEEVLNLAQSKNFHLRPRDLISNINVIVLELKGSETTFMCEYADETATIVEFLNRWITFCQSIISTLT

SEQ ID NO: 9 - protein, 119 aa, synthetic construct
  REGION 1..119: note = Variable heavy chain of anti-hCD73 Ab (CSA0060)
QVQLVQSGAEVKKPGSSVKVSCKFSGGSFTSYSFSWVRQAPGQGLEWMGRIIPVLTTTDYAQKFRDRVTITADESTSTAYMELSGLRSEDTAVYYCASGLKKNWYFDLWGRGALITVSS

SEQ ID NO: 10 - protein, 98 aa, synthetic construct
  REGION 1..98: note = Constant heavy chain of anti-hCD73 Ab (CSA0060)
ASTKGPSVFPLAPCSRSTSESTAALGCLVKDYFPEPVTVSWNSGALTSGVHTFPAVLQSSGLYSLSSVVTVPSSSLGTKTYTCNVDHKPSNTKVDKRV

SEQ ID NO: 11 - protein, 12 aa, synthetic construct
  REGION 1..12: note = Linker 3
ESKYGPPCPPCP

SEQ ID NO: 12 - protein, 10 aa, synthetic construct
  REGION 1..10: note = Linker 4
GGGGSGGGGS

SEQ ID NO: 13 - protein, 107 aa, synthetic construct
  REGION 1..107: note = Variable light chain of anti-hCD73 Ab (CSA0060)
DIQMTQSPSFLSASVGDRVTITCQASQDISHYLNWYQQKPGKAPKLLIYDASSLETGVPSRFSGSGSGTSFTLTISSLQPEDFATYYCQQYDDFPLTFGGGTKVDIK

SEQ ID NO: 14 - protein, 107 aa, synthetic construct
  REGION 1..107: note = Constant light chain of anti-hCD73 Ab (0060, kappa)
RSVAAPSVFIFPPSDEQLKSGTASVVCLLNNFYPREAKVQWKVDNALQSGNSQESVTEQDSKDSTYSLSSTLTLSKADYEKHKVYACEVTHQGLSSPVTKSFNRGEC

SEQ ID NO: 15 - protein, 8 aa, synthetic construct
  REGION 1..8: note = CDR1 of anti-hCD73 sdAb (AHF10235)
GRSISRYN

SEQ ID NO: 16 - protein, 8 aa, synthetic construct
  REGION 1..8: note = CDR2 of anti-hCD73 sdAb (AHF10235)
ISRSGGVT

SEQ ID NO: 17 - protein, 19 aa, synthetic construct
  REGION 1..19: note = CDR3 of anti-hCD73 sdAb (AHF10235)
AADWRNSDSPSPLIIVYDY

SEQ ID NO: 18 - protein, 8 aa, synthetic construct
  REGION 1..8: note = CDR1 of anti-hCD73 sdAb (AHF10240)
GRTFTHLA

SEQ ID NO: 19 - protein, 8 aa, synthetic construct
  REGION 1..8: note = CDR2 of anti-hCD73 sdAb (AHF10240)
ISNSGAGT

SEQ ID NO: 20 - protein, 19 aa, synthetic construct
  REGION 1..19: note = CDR3 of anti-hCD73 sdAb (AHF10240)
AADWGTRDSPSKLNAVYDY

SEQ ID NO: 21 - protein, 8 aa, synthetic construct
  REGION 1..8: note = CDR1 of anti-hCD73 sdAb (AHP04167)
GRTFSNYH

SEQ ID NO: 22 - protein, 8 aa, synthetic construct
  REGION 1..8: note = CDR2 of anti-hCD73 sdAb (AHP04167)
IGRSGGPT

SEQ ID NO: 23 - protein, 19 aa, synthetic construct
  REGION 1..19: note = CDR3 of anti-hCD73 sdAb (AHP04167)
AGDWRNSDSPSKLKPVYDY

SEQ ID NO: 24 - protein, 8 aa, synthetic construct
  REGION 1..8: note = VH-HCDR1 of anti-hCD73 Ab (CSA0060)
GGSFTSYS

SEQ ID NO: 25 - protein, 8 aa, synthetic construct
  REGION 1..8: note = VH-HCDR2 of anti-hCD73 sdAb (CSA0060)
IIPVLTTT

SEQ ID NO: 26 - protein, 11 aa, synthetic construct
  REGION 1..11: note = VH-HCDR3 of anti-hCD73 sdAb (CSA0060)
SGLKKNWYFDL

SEQ ID NO: 27 - protein, 6 aa, synthetic construct
  REGION 1..6: note = VL-LCDR1 of anti-hCD73 Ab (CSA0060)
QDISHY

SEQ ID NO: 28 - skipped

SEQ ID NO: 29 - protein, 8 aa, synthetic construct
  REGION 1..8: note = VL-LCDR3 of anti-hCD73 sdAb (CSA0060)
QYDDFPLT

SEQ ID NO: 30 - DNA, 1551 bp, synthetic construct
  misc_feature 1..1551: note = nucleotides coding for anti-hCD73 sdAb (AHF10235) conjugated withhIL2v3 and signal peptide
  source 1..1551: mol_type = other DNA
atggaatggtcctgggtgttcctgttcttcctgtccgtgaccaccggcgtgcactctcaggtgcaggttcaagaatctggcggcggattggtgcaggccggcgattctctgagactgtcttgtgccgcctctggccggtccatctctaggtacaacatgggctggttcagacaggcccctggcaaagagagagagttcgtcgccgccatcagcagatctggcggagtgacctactacgccgactccgtgaaaggccggctgaccatctccagagacaacgccaagtctgccgtgtacctccagatgaactccctgaagcctgaggacaccgccgtgtactactgtgccgccgattggcggaactccgactctccttctcctctgatcatcgtgtacgactactggggccagggcacccaagtgacagtttctagcggaggcggaggcagtgctgagtctaagtatggccctccttgtcctccatgtcctgctccagaagctgctggcgggccctccgtgtttctgttccctccaaagcctaaggaccagctgatgatctctcggacacccgaagtgacctgcgtggtggtggatgtgtctcaagaggaccctgaggtgcagttcaattggtacgtggacggcgtggaagtgcacaacgccaagaccaagcctagagaggaacagttcaactccacctacagagtggtgtccgtgctgaccgtgctgcaccaggattggctgaacggcaaagagtacaagtgcaaggtgtccaacaagggcctgccttccagcatcgaaaagaccatctccaaggccaagggccagcctagggaaccccaggtttacaccctgcctccaagccaagaggaaatgaccaagaaccaggtgtccctgacctgcctggtcaagggcttctacccttccgacattgccgtggaatgggagagcaatggccagcctgagaacaactacaagaccacacctcctgtgctggactccgacggctccttctttctgtactcccgcctgaccgtggacaagtccagatggcaagagggcaacgtgttctcctgctctgtgctgcacgaggccctgcacaatcactacacccagaagtccctcagcctgtcccttggcggaggcggtggatccgctcctacctccagctccaccaagaaaacccagttgcagctggaacatctgctgctggacctccagatgatcctgaatggcatcaacaattacaagaaccccaagctgaccgccatgctgaccgctaagttctacatgcccaagaaggccaccgagctgaagcacctccagtgcctggaacgggaactgaagcctctggaagaggtgctgaatctggcccagtccaagaacttccacctgaggcctcgggacctgatctccaacatcaacgtgatcgtgctggaactcaagggctccgagacaaccttcatgtgcgagtacgccgacgagacagctaccatcgtggaatttctgaatcggtggatcaccttctgccagtccatcatcagcaccctgacc

SEQ ID NO: 31 - DNA, 1494 bp, synthetic construct
  misc_feature 1..1494: note = nucleotides coding for anti-hCD73 sdAb (AHF10235) conjugated withhIL2v3
  source 1..1494: mol_type = other DNA
caggtgcaggttcaagaatctggcggcggattggtgcaggccggcgattctctgagactgtcttgtgccgcctctggccggtccatctctaggtacaacatgggctggttcagacaggcccctggcaaagagagagagttcgtcgccgccatcagcagatctggcggagtgacctactacgccgactccgtgaaaggccggctgaccatctccagagacaacgccaagtctgccgtgtacctccagatgaactccctgaagcctgaggacaccgccgtgtactactgtgccgccgattggcggaactccgactctccttctcctctgatcatcgtgtacgactactggggccagggcacccaagtgacagtttctagcggaggcggaggcagtgctgagtctaagtatggccctccttgtcctccatgtcctgctccagaagctgctggcgggccctccgtgtttctgttccctccaaagcctaaggaccagctgatgatctctcggacacccgaagtgacctgcgtggtggtggatgtgtctcaagaggaccctgaggtgcagttcaattggtacgtggacggcgtggaagtgcacaacgccaagaccaagcctagagaggaacagttcaactccacctacagagtggtgtccgtgctgaccgtgctgcaccaggattggctgaacggcaaagagtacaagtgcaaggtgtccaacaagggcctgccttccagcatcgaaaagaccatctccaaggccaagggccagcctagggaaccccaggtttacaccctgcctccaagccaagaggaaatgaccaagaaccaggtgtccctgacctgcctggtcaagggcttctacccttccgacattgccgtggaatgggagagcaatggccagcctgagaacaactacaagaccacacctcctgtgctggactccgacggctccttctttctgtactcccgcctgaccgtggacaagtccagatggcaagagggcaacgtgttctcctgctctgtgctgcacgaggccctgcacaatcactacacccagaagtccctcagcctgtcccttggcggaggcggtggatccgctcctacctccagctccaccaagaaaacccagttgcagctggaacatctgctgctggacctccagatgatcctgaatggcatcaacaattacaagaaccccaagctgaccgccatgctgaccgctaagttctacatgcccaagaaggccaccgagctgaagcacctccagtgcctggaacgggaactgaagcctctggaagaggtgctgaatctggcccagtccaagaacttccacctgaggcctcgggacctgatctccaacatcaacgtgatcgtgctggaactcaagggctccgagacaaccttcatgtgcgagtacgccgacgagacagctaccatcgtggaatttctgaatcggtggatcaccttctgccagtccatcatcagcaccctgacc

SEQ ID NO: 32 - DNA, 1551 bp, synthetic construct
  misc_feature 1..1551: note = nucleotides coding for anti-hCD73 sdAb (AHF10240) conjugated withhIL2v3 and signal peptide
  source 1..1551: mol_type = other DNA
atggaatggtcctgggtgttcctgttcttcctgtccgtgaccaccggcgtgcactctgaagtgcagctggttgaatctggcggcggagtggttcagacaggcggatctctgagactgtcttgtgccgcctccggcagaacctttacacacctggctatgggctggttccggcaggctcctggaaaagagagagagttcgtcgccgccatctccaactctggcgctggcacacagttcgccgactctgtgaagggcagattcaccatctctcgggacaacgccaagaacaccgtgtacctccagatgaactccctgaagcctgaggacaccgccgtgtactactgtgctgctgattggggcaccagagacagcccctctaagctgaatgccgtgtacgactactggggcagaggcacccaagtgacagtgtcctctggaggcggaggcagtgctgagtctaagtatggccctccttgtcctccatgtcctgctccagaagctgctggcgggccctccgtgtttctgttccctccaaagcctaaggaccagctgatgatctctcggacacccgaagtgacctgcgtggtggtggatgtgtctcaagaggaccctgaggtgcagttcaattggtacgtggacggcgtggaagtgcacaacgccaagaccaagcctagagaggaacagttcaactccacctacagagtggtgtccgtgctgaccgtgctgcaccaggattggctgaacggcaaagagtacaagtgcaaggtgtccaacaagggcctgccttccagcatcgaaaagaccatctccaaggccaagggccagcctagggaaccccaggtttacaccctgcctccaagccaagaggaaatgaccaagaaccaggtgtccctgacctgcctggtcaagggcttctacccttccgacattgccgtggaatgggagagcaatggccagcctgagaacaactacaagaccacacctcctgtgctggactccgacggctccttctttctgtactcccgcctgaccgtggacaagtccagatggcaagagggcaacgtgttctcctgctctgtgctgcacgaggccctgcacaatcactacacccagaagtccctcagcctgtcccttggcggaggcggtggatccgctcctacctccagctccaccaagaaaacccagttgcagctggaacatctgctgctggacctccagatgatcctgaatggcatcaacaattacaagaaccccaagctgaccgccatgctgaccgctaagttctacatgcccaagaaggccaccgagctgaagcacctccagtgcctggaacgggaactgaagcctctggaagaggtgctgaatctggcccagtccaagaacttccacctgaggcctcgggacctgatctccaacatcaacgtgatcgtgctggaactcaagggctccgagacaaccttcatgtgcgagtacgccgacgagacagctaccatcgtggaatttctgaatcggtggatcaccttctgccagtccatcatcagcaccctgacc

SEQ ID NO: 33 - DNA, 1494 bp, synthetic construct
  misc_feature 1..1494: note = nucleotides coding for anti-hCD73 sdAb (AHF10240) conjugated withhIL2v3
  source 1..1494: mol_type = other DNA
gaagtgcagctggttgaatctggcggcggagtggttcagacaggcggatctctgagactgtcttgtgccgcctccggcagaacctttacacacctggctatgggctggttccggcaggctcctggaaaagagagagagttcgtcgccgccatctccaactctggcgctggcacacagttcgccgactctgtgaagggcagattcaccatctctcgggacaacgccaagaacaccgtgtacctccagatgaactccctgaagcctgaggacaccgccgtgtactactgtgctgctgattggggcaccagagacagcccctctaagctgaatgccgtgtacgactactggggcagaggcacccaagtgacagtgtcctctggaggcggaggcagtgctgagtctaagtatggccctccttgtcctccatgtcctgctccagaagctgctggcgggccctccgtgtttctgttccctccaaagcctaaggaccagctgatgatctctcggacacccgaagtgacctgcgtggtggtggatgtgtctcaagaggaccctgaggtgcagttcaattggtacgtggacggcgtggaagtgcacaacgccaagaccaagcctagagaggaacagttcaactccacctacagagtggtgtccgtgctgaccgtgctgcaccaggattggctgaacggcaaagagtacaagtgcaaggtgtccaacaagggcctgccttccagcatcgaaaagaccatctccaaggccaagggccagcctagggaaccccaggtttacaccctgcctccaagccaagaggaaatgaccaagaaccaggtgtccctgacctgcctggtcaagggcttctacccttccgacattgccgtggaatgggagagcaatggccagcctgagaacaactacaagaccacacctcctgtgctggactccgacggctccttctttctgtactcccgcctgaccgtggacaagtccagatggcaagagggcaacgtgttctcctgctctgtgctgcacgaggccctgcacaatcactacacccagaagtccctcagcctgtcccttggcggaggcggtggatccgctcctacctccagctccaccaagaaaacccagttgcagctggaacatctgctgctggacctccagatgatcctgaatggcatcaacaattacaagaaccccaagctgaccgccatgctgaccgctaagttctacatgcccaagaaggccaccgagctgaagcacctccagtgcctggaacgggaactgaagcctctggaagaggtgctgaatctggcccagtccaagaacttccacctgaggcctcgggacctgatctccaacatcaacgtgatcgtgctggaactcaagggctccgagacaaccttcatgtgcgagtacgccgacgagacagctaccatcgtggaatttctgaatcggtggatcaccttctgccagtccatcatcagcaccctgacc

SEQ ID NO: 34 - DNA, 1551 bp, synthetic construct
  misc_feature 1..1551: note = nucleotides coding for anti-hCD73 sdAb (AHP04167) conjugated withhIL2v3 and signal peptide
  source 1..1551: mol_type = other DNA
atggaatggtcctgggtgttcctgttcttcctgtccgtgaccaccggcgtgcactctgaagtgcagctggttgaatctggcggcggattggttcaggctggcggatctctgagactgtcctgtgtggtgtccggcagaaccttctccaactaccacatgggctggttcagacaggcccctggcaaagaacgcgagttcgtggctgtgatcggcagatctggcggacctacctactacgccgactccgtgaagggcagattcaccatctccagagacaacgccaagaacaccgtgtacctccagatgaactccctgaagcctgaggacaccgccgtgtactactgtgccggcgattggagaaactccgactctcccagcaagctgaagcccgtgtacgattattggggccagggcacccaagtgaccgtgtcctctggaggcggaggcagtgctgagtctaagtatggccctccttgtcctccatgtcctgctccagaagctgctggcgggccctccgtgtttctgttccctccaaagcctaaggaccagctgatgatctctcggacacccgaagtgacctgcgtggtggtggatgtgtctcaagaggaccctgaggtgcagttcaattggtacgtggacggcgtggaagtgcacaacgccaagaccaagcctagagaggaacagttcaactccacctacagagtggtgtccgtgctgaccgtgctgcaccaggattggctgaacggcaaagagtacaagtgcaaggtgtccaacaagggcctgccttccagcatcgaaaagaccatctccaaggccaagggccagcctagggaaccccaggtttacaccctgcctccaagccaagaggaaatgaccaagaaccaggtgtccctgacctgcctggtcaagggcttctacccttccgacattgccgtggaatgggagagcaatggccagcctgagaacaactacaagaccacacctcctgtgctggactccgacggctccttctttctgtactcccgcctgaccgtggacaagtccagatggcaagagggcaacgtgttctcctgctctgtgctgcacgaggccctgcacaatcactacacccagaagtccctcagcctgtcccttggcggaggcggtggatccgctcctacctccagctccaccaagaaaacccagttgcagctggaacatctgctgctggacctccagatgatcctgaatggcatcaacaattacaagaaccccaagctgaccgccatgctgaccgctaagttctacatgcccaagaaggccaccgagctgaagcacctccagtgcctggaacgggaactgaagcctctggaagaggtgctgaatctggcccagtccaagaacttccacctgaggcctcgggacctgatctccaacatcaacgtgatcgtgctggaactcaagggctccgagacaaccttcatgtgcgagtacgccgacgagacagctaccatcgtggaatttctgaatcggtggatcaccttctgccagtccatcatcagcaccctgacc

SEQ ID NO: 35 - DNA, 1494 bp, synthetic construct
  misc_feature 1..1494: note = nucleotides coding for anti-hCD73 sdAb (AHP04167) conjugated withhIL2v3
  source 1..1494: mol_type = other DNA
gaagtgcagctggttgaatctggcggcggattggttcaggctggcggatctctgagactgtcctgtgtggtgtccggcagaaccttctccaactaccacatgggctggttcagacaggcccctggcaaagaacgcgagttcgtggctgtgatcggcagatctggcggacctacctactacgccgactccgtgaagggcagattcaccatctccagagacaacgccaagaacaccgtgtacctccagatgaactccctgaagcctgaggacaccgccgtgtactactgtgccggcgattggagaaactccgactctcccagcaagctgaagcccgtgtacgattattggggccagggcacccaagtgaccgtgtcctctggaggcggaggcagtgctgagtctaagtatggccctccttgtcctccatgtcctgctccagaagctgctggcgggccctccgtgtttctgttccctccaaagcctaaggaccagctgatgatctctcggacacccgaagtgacctgcgtggtggtggatgtgtctcaagaggaccctgaggtgcagttcaattggtacgtggacggcgtggaagtgcacaacgccaagaccaagcctagagaggaacagttcaactccacctacagagtggtgtccgtgctgaccgtgctgcaccaggattggctgaacggcaaagagtacaagtgcaaggtgtccaacaagggcctgccttccagcatcgaaaagaccatctccaaggccaagggccagcctagggaaccccaggtttacaccctgcctccaagccaagaggaaatgaccaagaaccaggtgtccctgacctgcctggtcaagggcttctacccttccgacattgccgtggaatgggagagcaatggccagcctgagaacaactacaagaccacacctcctgtgctggactccgacggctccttctttctgtactcccgcctgaccgtggacaagtccagatggcaagagggcaacgtgttctcctgctctgtgctgcacgaggccctgcacaatcactacacccagaagtccctcagcctgtcccttggcggaggcggtggatccgctcctacctccagctccaccaagaaaacccagttgcagctggaacatctgctgctggacctccagatgatcctgaatggcatcaacaattacaagaaccccaagctgaccgccatgctgaccgctaagttctacatgcccaagaaggccaccgagctgaagcacctccagtgcctggaacgggaactgaagcctctggaagaggtgctgaatctggcccagtccaagaacttccacctgaggcctcgggacctgatctccaacatcaacgtgatcgtgctggaactcaagggctccgagacaaccttcatgtgcgagtacgccgacgagacagctaccatcgtggaatttctgaatcggtggatcaccttctgccagtccatcatcagcaccctgacc

SEQ ID NO: 36 - DNA, 1806 bp, synthetic construct
  misc_feature 1..1806: note = nucleotides coding for heavy chain of anti-hCD73 (hIgG4Fc)conjugated with hIL2v3 and signal peptide
  source 1..1806: mol_type = other DNA
atggaatggtcctgggtgttcctgttcttcctgtccgtgaccaccggcgtgcactctcaggttcagttggttcagtctggcgccgaagtgaagaaacccggctcctctgtgaaggtgtcctgcaagttttccggcggctcctttacctcctacagcttctcctgggtccgacaggctcctggacaaggcttggagtggatgggcagaatcatccccgtgctgaccaccaccgattacgcccagaaattccgggacagagtgaccatcaccgccgacgagtctacctccaccgcctacatggaactgtccggcctgagatctgaggacaccgccgtgtactactgtgccagcggcctgaagaagaactggtacttcgacctgtggggcagaggcgctctgatcacagtgtcctccgcttccaccaagggacccagcgtgttccctctggctccttgctccagatccacctccgagtctacagctgctctgggctgtctggtcaaggactacttccctgagcctgtgaccgtgtcttggaactctggcgctctgacatctggcgtgcacacctttccagctgtgctccagtcctccggcctgtactctctgtctagcgtcgtgaccgtgccttcctctagcctgggcaccaagacctacacctgtaatgtggaccacaagccttccaacaccaaggtggacaagcgcgtggaatctaagtacggccctccttgtcctccatgtcctgctccagaagctgctggcggcccttccgtgtttctgttccctccaaagcctaaggaccagctgatgatctctcggacccctgaagtgacctgcgtggtggtggatgtgtcccaagaggaccctgaggtgcagttcaattggtacgtggacggcgtggaagtgcacaacgccaagaccaagcctagagaggaacagttcaactccacctacagagtggtgtccgtgctgaccgtgctgcaccaggattggctgaacggcaaagagtacaagtgcaaggtgtccaacaagggcctgccttccagcatcgaaaagaccatctctaaggctaagggccagcctcgcgagccccaggtttacacattgcctccaagccaagaggaaatgaccaagaaccaggtgtccctgacctgcctcgtgaagggcttctacccttccgacattgccgtggaatgggagtccaatggccagcctgagaacaactacaagacaacccctcctgtgctggactccgacggctccttctttctgtattcccgcctgaccgtggacaagtctaggtggcaagagggcaacgtgttctcctgctctgtgctgcacgaggccctgcacaatcactacacccagaagtctctgtctctgtcccttggcggaggcggaggatccgctcctacctccagctccaccaagaaaacccagttgcagctggaacatctgctgctggacctccagatgatcctgaatggcatcaacaattacaagaaccccaagctgaccgccatgctgaccgctaagttctacatgcccaagaaggccaccgagctgaagcacctccagtgcctggaacgggaactgaagcctctggaagaggtgctgaatctggcccagtccaagaacttccacctgaggcctcgggacctgatctccaacatcaacgtgatcgtgctggaactcaagggctccgagacaaccttcatgtgcgagtacgccgacgagacagctaccatcgtggaatttctgaatcggtggatcaccttctgccagtccatcatcagcaccctgacc

SEQ ID NO: 37 - DNA, 1749 bp, synthetic construct
  misc_feature 1..1749: note = nucleotides coding for heavy chain of anti-hCD73 (hIgG4Fc)conjugated with hIL2v3
  source 1..1749: mol_type = other DNA
caggttcagttggttcagtctggcgccgaagtgaagaaacccggctcctctgtgaaggtgtcctgcaagttttccggcggctcctttacctcctacagcttctcctgggtccgacaggctcctggacaaggcttggagtggatgggcagaatcatccccgtgctgaccaccaccgattacgcccagaaattccgggacagagtgaccatcaccgccgacgagtctacctccaccgcctacatggaactgtccggcctgagatctgaggacaccgccgtgtactactgtgccagcggcctgaagaagaactggtacttcgacctgtggggcagaggcgctctgatcacagtgtcctccgcttccaccaagggacccagcgtgttccctctggctccttgctccagatccacctccgagtctacagctgctctgggctgtctggtcaaggactacttccctgagcctgtgaccgtgtcttggaactctggcgctctgacatctggcgtgcacacctttccagctgtgctccagtcctccggcctgtactctctgtctagcgtcgtgaccgtgccttcctctagcctgggcaccaagacctacacctgtaatgtggaccacaagccttccaacaccaaggtggacaagcgcgtggaatctaagtacggccctccttgtcctccatgtcctgctccagaagctgctggcggcccttccgtgtttctgttccctccaaagcctaaggaccagctgatgatctctcggacccctgaagtgacctgcgtggtggtggatgtgtcccaagaggaccctgaggtgcagttcaattggtacgtggacggcgtggaagtgcacaacgccaagaccaagcctagagaggaacagttcaactccacctacagagtggtgtccgtgctgaccgtgctgcaccaggattggctgaacggcaaagagtacaagtgcaaggtgtccaacaagggcctgccttccagcatcgaaaagaccatctctaaggctaagggccagcctcgcgagccccaggtttacacattgcctccaagccaagaggaaatgaccaagaaccaggtgtccctgacctgcctcgtgaagggcttctacccttccgacattgccgtggaatgggagtccaatggccagcctgagaacaactacaagacaacccctcctgtgctggactccgacggctccttctttctgtattcccgcctgaccgtggacaagtctaggtggcaagagggcaacgtgttctcctgctctgtgctgcacgaggccctgcacaatcactacacccagaagtctctgtctctgtcccttggcggaggcggaggatccgctcctacctccagctccaccaagaaaacccagttgcagctggaacatctgctgctggacctccagatgatcctgaatggcatcaacaattacaagaaccccaagctgaccgccatgctgaccgctaagttctacatgcccaagaaggccaccgagctgaagcacctccagtgcctggaacgggaactgaagcctctggaagaggtgctgaatctggcccagtccaagaacttccacctgaggcctcgggacctgatctccaacatcaacgtgatcgtgctggaactcaagggctccgagacaaccttcatgtgcgagtacgccgacgagacagctaccatcgtggaatttctgaatcggtggatcaccttctgccagtccatcatcagcaccctgacc

SEQ ID NO: 38 - DNA, 699 bp, synthetic construct
  misc_feature 1..699: note = nucleotides coding for light chain of anti-hCD73 (hIgG4Fc)conjugated with hIL2v3 and signal peptide
  source 1..699: mol_type = other DNA
atggaatggtcctgggtgttcctgttcttcctgtccgtgaccaccggcgtgcactccgacattcagatgacccagtctccatccttcctgagcgcctctgtgggcgacagagtgaccattacctgtcaggccagccaggacatctcccactacctgaactggtatcagcagaagcccggcaaggcccctaagctgctgatctacgatgcctcctctctggaaactggcgtgccctccagattctccggctctggctctggcaccagctttaccctgaccatctctagcctccagcctgaggacttcgccacctactactgccagcagtacgacgacttcccactgacctttggcggaggcaccaaggtggacatcaagagatctgtggccgctccttccgtgttcatcttcccaccttccgacgagcagctgaagtccggcacagcttctgtcgtgtgcctgctgaacaacttctaccctcgggaagccaaggtgcagtggaaagtggataacgccctccagtccggcaactcccaagagtctgtgaccgagcaggactccaaggacagcacctacagcctgtcctccacactgaccctgtccaaggccgactacgagaagcacaaggtgtacgcctgcgaagtgacccatcagggcctgtctagccctgtgaccaagtctttcaaccggggcgagtgt

SEQ ID NO: 39 - DNA, 642 bp, synthetic construct
  misc_feature 1..642: note = nucleotides coding for light chain of anti-hCD73 (hIgG4Fc)conjugated with hIL2v3
  source 1..642: mol_type = other DNA
gacattcagatgacccagtctccatccttcctgagcgcctctgtgggcgacagagtgaccattacctgtcaggccagccaggacatctcccactacctgaactggtatcagcagaagcccggcaaggcccctaagctgctgatctacgatgcctcctctctggaaactggcgtgccctccagattctccggctctggctctggcaccagctttaccctgaccatctctagcctccagcctgaggacttcgccacctactactgccagcagtacgacgacttcccactgacctttggcggaggcaccaaggtggacatcaagagatctgtggccgctccttccgtgttcatcttcccaccttccgacgagcagctgaagtccggcacagcttctgtcgtgtgcctgctgaacaacttctaccctcgggaagccaaggtgcagtggaaagtggataacgccctccagtccggcaactcccaagagtctgtgaccgagcaggactccaaggacagcacctacagcctgtcctccacactgaccctgtccaaggccgactacgagaagcacaaggtgtacgcctgcgaagtgacccatcagggcctgtctagccctgtgaccaagtctttcaaccggggcgagtgt

SEQ ID NO: 40 - protein, 133 aa, synthetic construct [sequence omitted]

SEQ ID NO: 41 - protein, 574 aa, synthetic construct
  REGION 1..574: note = hCD73
MCPRAARAPATLLLALGAVLWPAAGAWELTILHTNDVHSRLEQTSEDSSKCVNASRCMGGVARLFTKVQQIRRAEPNVLLLDAGDQYQGTIWFTVYKGAEVAHFMNALRYDAMALGNHEFDNGVEGLIEPLLKEAKFPILSANIKAKGPLASQISGLYLPYKVLPVGDEVVGIVGYTSKETPFLSNPGTNLVFEDEITALQPEVDKLKTLNVNKIIALGHSGFEMDKLIAQKVRGVDVVVGGHSNTFLYTGNPPSKEVPAGKYPFIVTSDDGRKVPVVQAYAFGKYLGYLKIEFDERGNVISSHGNPILLNSSIPEDPSIKADINKWRIKLDNYSTQELGKTIVYLDGSSQSCRFRECNMGNLICDAMINNNLRHTDEMFWNHVSMCILNGGGIRSPIDERNNGTITWENLAAVLPFGGTFDLVQLKGSTLKKAFEHSVHRYGQSTGEFLQVGGIHVVYDLSRKPGDRVVKLDVLCTKCRVPSYDPLKMDEVYKVILPNFLANGGDGFQMIKDELLRHDSGDQDINVVSTYISKMKVIYPAVEGRIKFSTGSHCHGSFSLIFLSLWAVIFVLYQ

SEQ ID NO: 42 - DNA, 1392 bp, synthetic construct
  misc_feature 1..1392: note = nucleotides coding for heavy chain of anti-hCD73 (hIgG4Fc)conjugated with signal peptide
  source 1..1392: mol_type = other DNA
atggaatggtcctgggtgttcctgttcttcctgtccgtgaccaccggcgtgcactctcaggttcagttggttcagtctggcgccgaagtgaagaaacccggctcctctgtgaaggtgtcctgcaagttttccggcggctcctttacctcctacagcttctcctgggtccgacaggctcctggacaaggcttggagtggatgggcagaatcatccccgtgctgaccaccaccgattacgcccagaaattccgggacagagtgaccatcaccgccgacgagtctacctccaccgcctacatggaactgtccggcctgagatctgaggacaccgccgtgtactactgtgccagcggcctgaagaagaactggtacttcgacctgtggggcagaggcgctctgatcacagtgtcctccgcttccaccaagggacccagcgtgttccctctggctccttgctccagatccacctccgagtctacagctgctctgggctgtctggtcaaggactacttccctgagcctgtgaccgtgtcttggaactctggcgctctgacatctggcgtgcacacctttccagctgtgctccagtcctccggcctgtactctctgtctagcgtcgtgaccgtgccttcctctagcctgggcaccaagacctacacctgtaatgtggaccacaagccttccaacaccaaggtggacaagcgcgtggaatctaagtacggccctccttgtcctccatgtcctgctccagaagctgctggcggcccttccgtgtttctgttccctccaaagcctaaggaccagctgatgatctctcggacccctgaagtgacctgcgtggtggtggatgtgtcccaagaggaccctgaggtgcagttcaattggtacgtggacggcgtggaagtgcacaacgccaagaccaagcctagagaggaacagttcaactccacctacagagtggtgtccgtgctgaccgtgctgcaccaggattggctgaacggcaaagagtacaagtgcaaggtgtccaacaagggcctgccttccagcatcgaaaagaccatctctaaggctaagggccagcctcgcgagccccaggtttacacattgcctccaagccaagaggaaatgaccaagaaccaggtgtccctgacctgcctcgtgaagggcttctacccttccgacattgccgtggaatgggagtccaatggccagcctgagaacaactacaagacaacccctcctgtgctggactccgacggctccttctttctgtattcccgcctgaccgtggacaagtctaggtggcaagagggcaacgtgttctcctgctctgtgctgcacgaggccctgcacaatcactacacccagaagtctctgtctctgtcccttggc

SEQ ID NO: 43 - DNA, 1098 bp, synthetic construct
  misc_feature 1..1098: note = nucleotides coding for light chain of hIgG4Fc conjugated withhIL2v3 and signal peptide
  source 1..1098: mol_type = other DNA
gaatctaagtacggccctccttgtcctccatgtcctgctccagaagctgctggcggcccttccgtgtttctgttccctccaaagcctaaggaccagctgatgatctctcggacccctgaagtgacctgcgtggtggtggatgtgtcccaagaggaccctgaggtgcagttcaattggtacgtggacggcgtggaagtgcacaacgccaagaccaagcctagagaggaacagttcaactccacctacagagtggtgtccgtgctgaccgtgctgcaccaggattggctgaacggcaaagagtacaagtgcaaggtgtccaacaagggcctgccttccagcatcgaaaagaccatctctaaggctaagggccagcctcgcgagccccaggtttacacattgcctccaagccaagaggaaatgaccaagaaccaggtgtccctgacctgcctcgtgaagggcttctacccttccgacattgccgtggaatgggagtccaatggccagcctgagaacaactacaagacaacccctcctgtgctggactccgacggctccttctttctgtattcccgcctgaccgtggacaagtctaggtggcaagagggcaacgtgttctcctgctctgtgctgcacgaggccctgcacaatcactacacccagaagtctctgtctctgtcccttggcggaggcggaggatccgctcctacctccagctccaccaagaaaacccagttgcagctggaacatctgctgctggacctccagatgatcctgaatggcatcaacaattacaagaaccccaagctgaccgccatgctgaccgctaagttctacatgcccaagaaggccaccgagctgaagcacctccagtgcctggaacgggaactgaagcctctggaagaggtgctgaatctggcccagtccaagaacttccacctgaggcctcgggacctgatctccaacatcaacgtgatcgtgctggaactcaagggctccgagacaaccttcatgtgcgagtacgccgacgagacagctaccatcgtggaatttctgaatcggtggatcaccttctgccagtccatcatcagcaccctgacc